European Patent Application EP 4 741 423 A2, published May 13, 2026. Title: ANTIBODY-DRUG CONJUGATES AND THEIR USES. Applicant: MABLINK BIOSCIENCE. Application EP. The sequence listing filed with the application follows.

SEQUENCE LISTING (17 sequences)

SEQ ID NO: 1 - protein, 5 aa, synthetic construct
  REGION 1..5: note = Antibody
GYGLS

SEQ ID NO: 2 - protein, 17 aa, synthetic construct
  REGION 1..17: note = Antibody
MISSGGSYTYYADSVKG

SEQ ID NO: 3 - protein, 10 aa, synthetic construct
  REGION 1..10: note = Antibody
HGDDPAWFAY

SEQ ID NO: 4 - protein, 12 aa, synthetic construct
  REGION 1..12: note = Antibody
SVSSSISSNNLH

SEQ ID NO: 5 - protein, 7 aa, synthetic construct
  REGION 1..7: note = Antibody
GTSNLAS

SEQ ID NO: 6 - protein, 11 aa, synthetic construct
  REGION 1..11: note = Antibody
QQWSSYPYMYT

SEQ ID NO: 7 - protein, 119 aa, synthetic construct
  REGION 1..119: note = Antibody
EVQLVESGGGVVQPGRSLRLSCSASGFTFSGYGLSWVRQAPGKGLEWVAMISSGGSYTYYADSVKGRFAISRDNAKNTLFLQMDSLRPEDTGVYFCARHGDDPAWFAYWGQGTPVTVSS

SEQ ID NO: 8 - protein, 110 aa, synthetic construct
  REGION 1..110: note = Antibody
DIQLTQSPSSLSASVGDRVTITCSVSSSISSNNLHWYQQKPGKAPKPWIYGTSNLASGVPSRFSGSGSGTDYTFTISSLQPEDIATYYCQQWSSYPYMYTFGQGTKVEIK

SEQ ID NO: 9 - protein, 449 aa, synthetic construct
  REGION 1..449: note = Antibody
EVQLVESGGGVVQPGRSLRLSCSASGFTFSGYGLSWVRQAPGKGLEWVAMISSGGSYTYYADSVKGRFAISRDNAKNTLFLQMDSLRPEDTGVYFCARHGDDPAWFAYWGQGTPVTVSSASTKGPSVFPLAPSSKSTSGGTAALGCLVKDYFPEPVTVSWNSGALTSGVHTFPAVLQSSGLYSLSSVVTVPSSSLGTQTYICNVNHKPSNTKVDKKVEPKSCDKTHTCPPCPAPEAAGGPSVFLFPPKPKDTLMISRTPEVTCVVVDVSHEDPEVKFNWYVDGVEVHNAKTKPREEQYNSTYRVVSVLTVLHQDWLNGKEYKCKVSNKALPAPIEKTISKAKGQPREPQVYTLPPSRDELTKNQVSLTCLVKGFYPSDIAVEWESNGQPENNYKTTPPVLDSDGSFFLYSKLTVDKSRWQQGNVFSCSVMHEALHNHYTQKSLSLSPGK

SEQ ID NO: 10 - protein, 217 aa, synthetic construct
  REGION 1..217: note = Antibody
DIQLTQSPSSLSASVGDRVTITCSVSSSISSNNLHWYQQKPGKAPKPWIYGTSNLASGVPSRFSGSGSGTDYTFTISSLQPEDIATYYCQQWSSYPYMYTFGQGTKVEIKRTVAAPSVFIFPPSDEQLKSGTASVVCLLNNFYPREAKVQWKVDNALQSGNSQESVTEQDSKDSTYSLSSTLTLSKADYEKHKVYACEVTHQGLSSPVTKSFNRGEC

SEQ ID NO: 11 - protein, 449 aa, synthetic construct
  REGION 1..449: note = Antibody
EVQLVESGGGVVQPGRSLRLSCSASGFTFSGYGLSWVRQAPGKGLEWVAMISSGGSYTYYADSVKGRFAISRDNAKNTLFLQMDSLRPEDTGVYFCARHGDDPAWFAYWGQGTPVTVSSASTKGPSVFPLAPSSKSTSGGTAALGCLVKDYFPEPVTVSWNSGALTSGVHTFPAVLQSSGLYSLSSVVTVPSSSLGTQTYICNVNHKPSNTKVDKKVEPKSCDKTHTCPPCPAPELLGGPSVFLFPPKPKDTLMISRTPEVTCVVVDVSHEDPEVKFNWYVDGVEVHNAKTKPREEQYNSTYRVVSVLTVLHQDWLNGKEYKCKVSNKALPAPIEKTISKAKGQPREPQVYTLPPSRDELTKNQVSLTCLVKGFYPSDIAVEWESNGQPENNYKTTPPVLDSDGSFFLYSKLTVDKSRWQQGNVFSCSVMHEALHNHYTQKSLSLSPGK

SEQ ID NO: 12 - protein, 257 aa, Homo sapiens
MAQRMTTQLLLLLVWVAVVGEAQTRIAWARTELLNVCMNAKHHKEKPGPEDKLHEQCRPWRKNACCSTNTSQEAHKDVSYLYRFNWNHCGEMAPACKRHFIQDTCLYECSPNLGPWIQQVDQSWRKERVLNVPLCKEDCEQWWEDCRTSYTCKSNWHKGWNWTSGFNKCAVGAACQPFHFYFPTPTVLCNEIWTHSYKVSNYSRGSGRCIQMWFDPAQGNPNEEVARFYAAAMSGAGPWAAWPFLLSLALMLLWLLS

SEQ ID NO: 13 - DNA, 1428 bp, synthetic construct
  misc_feature 1..1428: note = Antibody
  source 1..1428: mol_type = other DNA
gcggccgccatgaattttggactgaggctgattttcctggtgctgaccctgaaaggcgtccagtgtgaagtccaattagtcgagagtggcgggggggtcgtccaacccggccgttcattacggctctcctgctccgcctctgggttcaccttctcggggtacggcctatcatgggtccgtcaagctcctggcaaaggcctggaatgggtcgccatgattagtagcggggggagctatacctattacgccgacagtgtgaaggggcgattcgccattagtagggacaatgcaaagaacacgctgtttctgcaaatggactcgttgagacccgaggacacgggtgtctacttttgcgcacgtcacggtgacgatccagcctggttcgcatattgggggcagggtacccccgttacggtctcgagcgctagcacaaagggccctagtgtgtttcctctggctccctcttccaaatccacttctggtggcactgctgctctgggatgcctggtgaaggattactttcctgaacctgtgactgtctcatggaactctggtgctctgacttctggtgtccacactttccctgctgtgctgcagtctagtggactgtactctctgtcatctgtggtcactgtgccctcttcatctctgggaacccagacctacatttgtaatgtgaaccacaaaccatccaacactaaagtggacaaaaaagtggaacccaaatcctgtgacaaaacccacacctgcccaccttgtcctgcccctgaagccgccggaggaccttctgtgtttctgttcccccccaaaccaaaggataccctgatgatctctagaacccctgaggtgacatgtgtggtggtggatgtgtctcatgaggaccctgaggtcaaattcaactggtacgtggatggagtggaagtccacaatgccaaaaccaagcctagagaggaacagtacaattcaacctacagagtggtcagtgtgctgactgtgctgcatcaggattggctgaatggcaaggaatacaagtgtaaagtctcaaacaaggccctgcctgctccaattgagaaaacaatctcaaaggccaagggacagcctagggaaccccaggtctacaccctgccaccttcaagagacgaactgaccaaaaaccaggtgtccctgacatgcctggtcaaaggcttctacccttctgacattgctgtggagtgggagtcaaatggacagcctgagaacaactacaaaacaaccccccctgtgctggattctgatggctctttctttctgtactccaaactgactgtggacaagtctagatggcagcaggggaatgtcttttcttgctctgtcatgcatgaggctctgcataaccactacactcagaaatccctgtctctgtctcccgggaaatgatagtaaaagctt

SEQ ID NO: 14 - DNA, 732 bp, synthetic construct
  misc_feature 1..732: note = Antibody
  source 1..732: mol_type = other DNA
gcggccgccatgaattttggactgaggctgattttcctggtgctgaccctgaaaggcgtccagtgtgacatccagctgacacagagcccaagttccctgtctgcatccgtgggggatagggttacaatcacttgtagtgtaagcagctcgatcagcagcaataacctgcactggtatcaacagaaaccgggtaaggcaccaaagccttggatttacggcaccagtaatctggcctccggggtgccgtctcgcttttctgggtccggcagcggtactgactacacatttacaatcagcagcctacagcctgaggacattgcgacctattactgccagcagtggtccagctacccatatatgtatacgttcgggcagggtaccaaggtcgagatcaagcgtacggtcgcggcgccttctgtgttcattttccccccatctgatgaacagctgaaatctggcactgcttctgtggtctgtctgctgaacaacttctaccctagagaggccaaagtccagtggaaagtggacaatgctctgcagagtgggaattcccaggaatctgtcactgagcaggactctaaggatagcacatactccctgtcctctactctgacactgagcaaggctgattacgagaaacacaaagtgtacgcctgtgaagtcacacatcaggggctgtctagtcctgtgaccaaatccttcaataggggagagtgctgatagtaaaagctt

SEQ ID NO: 15 - DNA, 1428 bp, synthetic construct
  misc_feature 1..1428: note = Antibody
  source 1..1428: mol_type = other DNA
gcggccgccatgaattttggactgaggctgattttcctggtgctgaccctgaaaggcgtccagtgtgaagtccaattagtcgagagtggcgggggggtcgtccaacccggccgttcattacggctctcctgctccgcctctgggttcaccttctcggggtacggcctatcatgggtccgtcaagctcctggcaaaggcctggaatgggtcgccatgattagtagcggggggagctatacctattacgccgacagtgtgaaggggcgattcgccattagtagggacaatgcaaagaacacgctgtttctgcaaatggactcgttgagacccgaggacacgggtgtctacttttgcgcacgtcacggtgacgatccagcctggttcgcatattgggggcagggtacccccgttacggtctcgagcgctagcacaaagggccctagtgtgtttcctctggctccctcttccaaatccacttctggtggcactgctgctctgggatgcctggtgaaggattactttcctgaacctgtgactgtctcatggaactctggtgctctgacttctggtgtccacactttccctgctgtgctgcagtctagtggactgtactctctgtcatctgtggtcactgtgccctcttcatctctgggaacccagacctacatttgtaatgtgaaccacaaaccatccaacactaaagtggacaaaaaagtggaacccaaatcctgtgacaaaacccacacctgcccaccttgtcctgcccctgaactgctgggaggaccttctgtgtttctgttcccccccaaaccaaaggataccctgatgatctctagaacccctgaggtgacatgtgtggtggtggatgtgtctcatgaggaccctgaggtcaaattcaactggtacgtggatggagtggaagtccacaatgccaaaaccaagcctagagaggaacagtacaattcaacctacagagtggtcagtgtgctgactgtgctgcatcaggattggctgaatggcaaggaatacaagtgtaaagtctcaaacaaggccctgcctgctccaattgagaaaacaatctcaaaggccaagggacagcctagggaaccccaggtctacaccctgccaccttcaagagacgaactgaccaaaaaccaggtgtccctgacatgcctggtcaaaggcttctacccttctgacattgctgtggagtgggagtcaaatggacagcctgagaacaactacaaaacaaccccccctgtgctggattctgatggctctttctttctgtactccaaactgactgtggacaagtctagatggcagcaggggaatgtcttttcttgctctgtcatgcatgaggctctgcataaccactacactcagaaatccctgtctctgtctcccgggaaatgatagtaaaagctt

SEQ ID NO: 16 - protein, 447 aa, synthetic construct
  REGION 1..447: note = Antibody
QVQLVQSGAEVVKPGASVKISCKASGYTFTGYFMNWVKQSPGQSLEWIGRIHPYDGDTFYNQKFQGKATLTVDKSSNTAHMELLSLTSEDFAVYYCTRYDGSRAMDYWGQGTTVTVSSASTKGPSVFPLAPSSKSTSGGTAALGCLVKDYFPEPVTVSWNSGALTSGVHTFPAVLQSSGLYSLSSVVTVPSSSLGTQTYICNVNHKPSNTKVDKKVEPKSCDKTHTCPPCPAPELLGGPSVFLFPPKPKDTLMISRTPEVTCVVVDVSHEDPEVKFNWYVDGVEVHNAKTKPREEQYNSTYRVVSVLTVLHQDWLNGKEYKCKVSNKALPAPIEKTISKAKGQPREPQVYTLPPSRDELTKNQVSLTCLVKGFYPSDIAVEWESNGQPENNYKTTPPVLDSDGSFFLYSKLTVDKSRWQQGNVFSCSVMHEALHNHYTQKSLSLSPG

SEQ ID NO: 17 - protein, 218 aa, synthetic construct
  REGION 1..218: note = Antibody
DIVLTQSPLSLAVSLGQPAIISCKASQSVSFAGTSLMHWYHQKPGQQPRLLIYRASNLEAGVPDRFSGSGSKTDFTLTISPVEAEDAATYYCQQSREYPYTFGGGTKLEIKRTVAAPSVFIFPPSDEQLKSGTASVVCLLNNFYPREAKVQWKVDNALQSGNSQESVTEQDSKDSTYSLSSTLTLSKADYEKHKVYACEVTHQGLSSPVTKSFNRGEC